European Patent Specification EP 3 128 842 B1, published July 26, 2023. Title: COH29 TREATMENT OF BRCA1-DEFECTIVE CANCER OR RESISTANT CANCERS. Applicant: City of Hope Yen, Yun. The sequence listing filed with the application follows.

SEQUENCE LISTING (4 sequences)

SEQ ID NO: 1 - RNA, 19 nt, Artificial sequence
  Synthetic polynucleotide
ucacaguguccuuuaugua

SEQ ID NO: 2 - RNA, 19 nt, Artificial sequence
  Synthetic polynucleotide
uacauaaaggacacuguga

SEQ ID NO: 3 - DNA, 24 bp, Artificial sequence
  Synthetic polynucleotide
aggaattgcgggaggaaaatgggt

SEQ ID NO: 4 - DNA, 24 bp, Artificial sequence
  Synthetic polynucleotide
gccccctgaagatctttctgtcct